European Patent Specification EP 3 390 643 B1, published June 28, 2023. Title: PLASMID CONSTRUCTS FOR HETEROLOGOUS PROTEIN EXPRESSION AND METHODS OF USE. Applicant: Campbell, Jean Canton, David A. Pierce, Robert H. The sequence listing filed with the application follows.

SEQUENCE LISTING (25 sequences)

SEQ ID NO: 1 - DNA, 576 bp, Artificial Sequence
  Human CMV promoter/enhancer
tagtaatcaattacggggtcattagttcatagcccatatatggagttccgcgttacataacttacggtaaatggcccgcctggctgaccgcccaacgacccccgcccattgacgtcaataatgacgtatgttcccatagtaacgccaatagggactttccattgacgtcaatgggtggagtatttacggtaaactgcccacttggcagtacatcaagtgtatcatatgccaagtacgccccctattgacgtcaatgacggtaaatggcccgcctggcattatgcccagtacatgaccttatgggactttcctacttggcagtacatctacgtattagtcatcgctattaccatggtgatgcggttttggcagtacatcaatgggcgtggatagcggtttgactcacggggatttccaagtctccaccccattgacgtcaatgggagtttgttttggcaccaaaatcaacgggactttccaaaatgtcgtaacaactccgccccattgacgcaaatgggcggtaggcgtgtacggtgggaggtctatataagcagagctcgtttagtgaaccgtcag

SEQ ID NO: 2 - DNA, 593 bp, Artificial Sequence
  Simian CMV promoter/enhancer
atagtattccatatatgggttttcctattgacgtagatagcccctcccaatgggcggtcccatataccatatatggggcttcctaataccgcccatagccactcccccattgacgtcaatggtctctatatatggtctttttcgaacctattgacgtcatatgggcggtcctattgacgtatatggcgcctcccccattgacgtcaattacggtaaatggcccgcctggctcaatgcccattgacgtcaataggaccacccaccattgacgtcaatgggatggctcattgcccattcatatccgttctcacgccccctattgacgtcaatgacggtaaatggcccacttggcagtacatcaatatctattaatagtaacttggcaagtacattactattggaagtacgccagggtacattggcagtactcccattgacgtcaatggcggtaaatggcccgcgatggctgccaagtacatccccattgacgtcaatggggaggggcaatgacgcaaatgggcgttccattgacgtaaatgggcggtaggcgtgcctaatgggaggtctatataagcaatgctcgtttagggaac

SEQ ID NO: 3 - DNA, 511 bp, Mus musculus
ttctaccgggtaggggaggcgcttttcccaaggcagtctggagcatgcgctttagcagccccgctgggcacttggcgctacacaagtggcctctggcctcgcacacattccacatccaccggtaggcgccaaccggctccgttctttggtggccccttcgcgccaccttctactcctcccctagtcaggaagttcccccccgccccgcagctcgcgtcgtgcaggacgtgacaaatggaagtagcacgtctcactagtctcgtgcagatggacagcaccgctgagcaatggaagcgggtaggcctttggggcagcggccaatagcagctttgctccttcgctttctgggctcagaggctgggaaggggtgggtccgggggcgggctcaggggcgggctcaggggcggggcgggcgcccgaaggtcctccggaggcccggcattctgcacgcttcaaaagcgcacgtctgccgcgctgttctcctcttcctcatctccgggcctttcgacct

SEQ ID NO: 4 - DNA, 344 bp, Artificial Sequence
  SV-40 promoter
ctgtggaatgtgtgtcagttagggtgtggaaagtccccaggctccccagcaggcagaagtatgcaaagcatgcatctcaattagtcagcaaccaggtgtggaaagtccccaggctccccagcaggcagaagtatgcaaagcatgcatctcaattagtcagcaaccatagtcccgcccctaactccgcccatcccgcccctaactccgcccagttccgcccattctccgccccatggctgactaattttttttatttatgcagaggccgaggccgcctctgcctctgagctattccagaagtagtgaggaggcttttttggaggcctaggcttttgcaaaaagct

SEQ ID NO: 5 - DNA, 1824 bp, Artificial Sequence
  Human IL12p35-P2A-IL12p40
atgtggccccctgggtcagcctcccagccaccgccctcacctgccgcggccacaggtctgcatccagcggctcgccctgtgtccctgcagtgccggctcagcatgtgtccagcgcgcagcctcctccttgtggctaccctggtcctcctggaccacctcagtttggccagaaacctccccgtggccactccagacccaggaatgttcccatgccttcaccactcccaaaacctgctgagggccgtcagcaacatgctccagaaggccagacaaactctcgaattttacccttgcacttctgaagagattgatcatgaagatatcacaaaagataaaaccagcacagtggaggcctgtttaccattggaattaaccaagaatgagagttgcctaaattccagagagacctctttcataactaatgggagttgcctggcctccagaaagacctcttttatgatggccctgtgccttagtagtatttatgaagacttgaagatgtaccaggtggagttcaagaccatgaatgcaaagcttctgatggaccctaagaggcaaatcttcctagatcaaaacatgctggcagttattgatgagctgatgcaggccctgaatttcaacagtgagactgtgccacaaaaatcctcccttgaagaaccggatttctacaagactaaaatcaagctctgcatacttcttcatgctttcagaattcgggcagtgactattgatagagtgatgagctatctgaatgcttccgcggccgcaggatctggggccaccaacttttcattgctcaagcaggcgggcgatgtggaggaaaaccctggccccggatcctgtcaccagcagttggtcatctcttggttttccctggtttttctggcatctcccctcgtggccatatgggaactgaagaaagatgtttatgtcgtagaattggattggtatccggatgcccctggagaaatggtggtcctcacctgtgacacccctgaagaagatggtatcacctggaccttggaccagagcagtgaggtcttaggctctggcaaaaccctgaccatccaagtcaaagagtttggagatgctggccagtacacctgtcacaaaggaggcgaggttctaagccattcgctcctgctgcttcacaaaaaggaagatggaatttggtccactgatattttaaaggaccagaaagaacccaaaaataagacctttctaagatgcgaggccaagaattattctggacgtttcacctgctggtggctgacgacaatcagtactgatttgacattcagtgtcaaaagcagcagaggctcttctgacccccaaggggtgacgtgcggagctgctacactctctgcagagagagtcagaggggacaacaaggagtatgagtactcagtggagtgccaggaggacagtgcctgcccagctgctgaggagagtctgcccattgaggtcatggtggatgccgttcacaagctcaagtatgaaaactacaccagcagcttcttcatcagggacatcatcaaacctgacccacccaagaacttgcagctgaagccattaaagaattctcggcaggtggaggtcagctgggagtaccctgacacctggagtactccacattcctacttctccctgacattctgcgttcaggtccagggcaagagcaagagagaaaagaaagatagagtcttcacggacaagacctcagccacggtcatctgccgcaaaaatgccagcattagcgtgcgggcccaggaccgctactatagctcatcttggagcgaatgggcatctgtgccctgcagttag

SEQ ID NO: 6 - DNA, 1794 bp, Artificial Sequence
  Mouse IL12p35-P2A-IL12p40
atggtcagcgttccaacagcctcaccctcggcatccagcagctcctctcagtgccggtccagcatgtgtcaatcacgctacctcctctttttggccacccttgccctcctaaaccacctcagtttggccagggtcattccagtctctggacctgccaggtgtcttagccagtcccgaaacctgctgaagaccacagatgacatggtgaagacggccagagaaaaactgaaacattattcctgcactgctgaagacatcgatcatgaagacatcacacgggaccaaaccagcacattgaagacctgtttaccactggaactacacaagaacgagagttgcctggctactagagagacttcttccacaacaagagggagctgcctgcccccacagaagacgtctttgatgatgaccctgtgccttggtagcatctatgaggacttgaagatgtaccagacagagttccaggccatcaacgcagcacttcagaatcacaaccatcagcagatcattcttgacaagggcatgctggtggccatcgatgagctgatgcagtctctgaatcataatggcgagactctgcgccagaaacctcctgtgggagaagcagacccttacagagtgaaaatgaagctctgcatcctgcttcacgccttcagcacccgcgtcgtgaccatcaacagggtgatgggctatctgagctccgccgcggccgcaggatctggggccaccaacttttcattgctcaagcaggcgggcgatgtggaggaaaaccctggccccggatcctgtcctcagaagctaaccatctcctggtttgccatcgttttgctggtgtctccactcatggccatgtgggagctggagaaagacgtttatgttgtagaggtggactggactcccgatgcccctggagaaacagtgaacctcacctgtgacacgcctgaagaagatgacatcacctggacctcagaccagagacatggagtcataggctctggaaagaccctgaccatcactgtcaaagagtttcttgatgctggccagtacacctgccacaaaggaggcgagactctgagccactcacatctgctgctccacaagaaggaaaatggaatttggtccactgaaattttaaagaatttcaagaacaagactttcctgaagtgtgaagcaccaaattactccggacggttcacgtgctcatggctggtgcaaagaaacatggacttgaagttcaacatcaagagcagtagcagttcccctgactctcgggcagtgacatgtggaatggcgtctctgtctgcagagaaggtcacactggaccaaagggactatgagaagtattcagtgtcctgccaggaggatgtcacctgcccaactgccgaggagaccctgcccattgaactggcgttggaagcacggcagcagaataaatatgagaactacagcaccagcttcttcatcagggacatcatcaaaccagacccgcccaagaacttgcagatgaagcctttgaagaactcacaggtggaggtcagctgggagtaccctgactcctggagcactccccattcctacttctccctcaagttctttgttcgaatccagcgcaagaaagaaaagatgaaggagacagaggaggggtgtaaccagaaaggtgcgttcctcgtagagaagacatctaccgaagtccaatgcaaaggcgggaatgtctgcgtgcaagctcaggatcgctattacaattcctcatgcagcaagtgggcatgtgttccctgcagggtccgatcctag

SEQ ID NO: 7 - DNA, 1734 bp, Artificial Sequence
  Canine IL12p35-P2A-IL12p40
atgtgcccgccgcgcggcctcctccttgtgaccatcctggtcctgctaagccacctggaccaccttacttgggccaggagcctccccacagcctcaccgagcccaggaatattccagtgcctcaaccactcccaaaacctgctgagagccgtcagcaacacgcttcagaaggccagacaaactctcgattatattccctgcacttccgaagagattgatcatgaagatatcacaaaggataaaaccagcacagtggaggcctgcttaccactggaattaaccatgaatgagagttgcctggcttccagagagatttctttgataactaacgggagttgcctggcctctggaaaggcctcttttatgacggtcctgtgccttagcagcatctatgaggacttgaagatgtaccagatggaattcaaggccatgaacgcaaagcttttaatggaccccaagaggcagatttttctggatcaaaacatgttgacagctatcgatgagctgttacaggccctgaatttcaacagtgtgactgtgccacagaaatcctcccttgaagagccggacttctacaagactaaaatcaagctctgcatacttcttcatgctttcagaattcgtgcggtgaccatcgatagaatgatgagttatctgaattcttccgcggccgcaggatctggggccaccaacttttcattgctcaagcaggcgggcgatgtggaggaaaaccctggccccggatcccatcctcagcagttggtcatctcctggttttccctcgttttgctggcgtcttccctcatgaccatatgggaactggagaaagatgtttatgttgtagagttggactggcaccctgatgcccccggagaaatggtggtcctcacctgccatacccctgaagaagatgacatcacttggacctcagcgcagagcagtgaagtcctaggttctggtaaaactctgaccatccaagtcaaagaatttggagatgctggccagtatacctgccataaaggaggcaaggttctgagccgctcactcctgttgattcacaaaaaagaagatggaatttggtccactgatatcttaaaggaacagaaagaatccaaaaataagatttttctgaaatgtgaggcaaagaattattctggacgtttcacatgctggtggctgacggcaatcagtactgatttgaaattcagtgtcaaaagtagcagaggcttctctgacccccaaggggtgacatgtggagcagtgacactttcagcagagagggtcagagtggacaacagggattataagaagtacacagtggagtgtcaggaaggcagtgcctgcccctctgccgaggagagcctacccatcgaggtcgtggtggatgctattcacaagctcaagtatgaaaactacaccagcagcttcttcatcagagacatcatcaaaccagacccacccacaaacctgcagctgaagccattgaaaaattctcggcacgtggaggtcagctgggaataccccgacacctggagcaccccacattcctacttctccctgacattttgcgtacaggcccagggcaagaacaatagagaaaagaaagatagactctgcgtggacaagacctcagccaaggtcgtgtgccacaaggatgccaagatccgcgtgcaagcccgagaccgctactatagttcatcctggagcgactgggcatctgtgtcctgcagttag

SEQ ID NO: 8 - DNA, 1368 bp, Artificial Sequence
  Human IL-15/IL-15Ra with P2A
atgagaatttcgaaaccacatttgagaagtatttccatccagtgctacttgtgtttacttctaaacagtcattttctaactgaagctggcattcatgtcttcattttgggctgtttcagtgcagggcttcctaaaacagaagccaactgggtgaatgtaataagtgatttgaaaaaaattgaggatcttattcaatctatgcatattgatgctactttatatacggaaagtgatgttcaccccagttgcaaagtaacagcaatgaagtgctttctcttggagttacaagttatttcacttgagtccggagatgcaagtattcatgatacagtagaaaatctgatcatcctagcaaacaacagtttgtcttctaatgggaatgtaacagaatctggatgcaaagaatgtgaggaactggaggaaaagaatattaaagagtttttgcagagttttgtacatattgtccaaatgttcatcaacacttctgcggccgcaggatctggggccaccaacttttcattgctcaagcaggcgggcgatgtggaggaaaaccctggccccggatccgctccccgccgcgcgagagggtgtcgaacgcttggtcttcctgcgttgctgctgttgttgttgctcaggccgcctgccacccgcggcataacctgccccccaccgatgagcgtggagcacgcagacatctgggtcaaaagctatagtctgtactctagggaaaggtacatttgtaacagtgggttcaaaagaaaggctggcacatcatcccttacagaatgcgtccttaacaaggccaccaacgtcgcgcattggactaccccttccctgaagtgcatcagagatcctgcgctggttcaccaacgcccggcccccccatctacagttacaaccgctggtgttacacctcagcccgaatctctgtcaccttctggcaaagaaccagcagcctcctccccaagttccaacaataccgccgccactaccgctgctatcgttccaggctcacaactgatgccgagtaaatctcccagcaccggtacaacagaaatctctagtcatgagtcctcccatgggaccccgtcccagaccactgctaaaaactgggagctgaccgcctccgctagccatcagccgcccggggtgtacccacaggggcactctgacaccactgtcgcgattagtactagcacagtgctgttgtgcggactgtctgccgtcagcttgttggcttgctatctgaaatcccggcagacgccaccactggccagcgtggagatggaagcaatggaagctttgcctgtaacctgggggacgagctcacgggatgaggatctggagaactgctcacatcacctgtaa

SEQ ID NO: 9 - protein, 455 aa, Artificial Sequence
  Human IL-15/IL-15Ra Fc P2A
MRISKPHLRSISIQCYLCLLLNSHFLTEAGIHVFILGCFSAGLPKTEANWVNVISDLKKIEDLIQSMHIDATLYTESDVHPSCKVTAMKCFLLELQVISLESGDASIHDTVENLIILANNSLSSNGNVTESGCKECEELEEKNIKEFLQSFVHIVQMFINTSAAAGSGATNFSLLKQAGDVEENPGPGSAPRRARGCRTLGLPALLLLLLLRPPATRGITCPPPMSVEHADIWVKSYSLYSRERYICNSGFKRKAGTSSLTECVLNKATNVAHWTTPSLKCIRDPALVHQRPAPPSTVTTAGVTPQPESLSPSGKEPAASSPSSNNTAATTAAIVPGSQLMPSKSPSTGTTEISSHESSHGTPSQTTAKNWELTASASHQPPGVYPQGHSDTTVAISTSTVLLCGLSAVSLLACYLKSRQTPPLASVEMEAMEALPVTWGTSSRDEDLENCSHHL

SEQ ID NO: 10 - DNA, 2070 bp, Artificial Sequence
  Human IL-15/IL-15Ra-Fc with P2A
atgagaatttcgaaaccacatttgagaagtatttccatccagtgctacttgtgtttacttctaaacagtcattttctaactgaagctggcattcatgtcttcattttgggctgtttcagtgcagggcttcctaaaacagaagccaactgggtgaatgtaataagtgatttgaaaaaaattgaggatcttattcaatctatgcatattgatgctactttatatacggaaagtgatgttcaccccagttgcaaagtaacagcaatgaagtgctttctcttggagttacaagttatttcacttgagtccggagatgcaagtattcatgatacagtagaaaatctgatcatcctagcaaacaacagtttgtcttctaatgggaatgtaacagaatctggatgcaaagaatgtgaggaactggaggaaaagaatattaaagagtttttgcagagttttgtacatattgtccaaatgttcatcaacacttctgcggccgcaggatctggggccaccaacttttcattgctcaagcaggcgggcgatgtggaggaaaaccctggccccggatccgctccccgccgcgcgagagggtgtcgaacgcttggtcttcctgcgttgctgctgttgttgttgctcaggccgcctgccacccgcggcataacctgccccccaccgatgagcgtggagcacgcagacatctgggtcaaaagctatagtctgtactctagggaaaggtacatttgtaacagtgggttcaaaagaaaggctggcacatcatcccttacagaatgcgtccttaacaaggccaccaacgtcgcgcattggactaccccttccctgaagtgcatcagagatcctgcgctggttcaccaacgcccggcccccccatctacagttacaaccgctggtgttacacctcagcccgaatctctgtcaccttctggcaaagaaccagcagcctcctccccaagttccaacaataccgccgccactaccgctgctatcgttccaggctcacaactgatgccgagtaaatctcccagcaccggtacaacagaaatctctagtcatgagtcctcccatgggaccccgtcccagaccactgctaaaaactgggagctgaccgcctccgctagccatcagccgcccggggtgtacccacaggggcactctgacaccactgtcgcgattagtactagcacagtgctgttgtgcggactgtctgccgtcagcttgttggcttgctatctgaaatcccggcagacgccaccactggccagcgtggagatggaagcaatggaagctttgcctgtaacctgggggacgagctcacgggatgaggatctggagaactgctcacatcacctgggaagatctggcagttctggggacaaaactcacacatgcccaccgtgcccagcacctgaactcctggggggaccgtcagtcttcctcttccccccaaaacccaaggacaccctcatgatctcccggacccctgaggtcacatgcgtggtggtggacgtgagccacgaagaccctgaggtcaagttcaactggtacgtggacggcgtggaggtgcataatgccaagacaaagccgcgggaggagcagtacaacagcacgtaccgtgtggtcagcgtcctcaccgtcctgcaccaggactggctgaatggcaaggagtacaagtgcaaggtctccaacaaagccctcccagcccccatcgagaaaaccatctccaaagccaaagggcagccccgagaaccacaggtctacaccctgcccccatcccgggaggagatgaccaagaaccaggtcagcctgacctgcctggtcaaaggcttctatcccagcgacatcgccgtggagtgggagagcaatgggcagccggagaacaactacaagaccacgcctcccgtgctggactccgacggctccttcttcctctacagcaagctcaccgtggacaagagcaggtggcagcaggggaacgtcttctcatgctccgtgatgcacgaggctctgcacaaccactacacgcagaagagcctctccctgtctccgggtaaatag

SEQ ID NO: 11 - protein, 689 aa, Artificial Sequence
  Human IL-15/IL-15Ra-Fc with P2A
MRISKPHLRSISIQCYLCLLLNSHFLTEAGIHVFILGCFSAGLPKTEANWVNVISDLKKIEDLIQSMHIDATLYTESDVHPSCKVTAMKCFLLELQVISLESGDASIHDTVENLIILANNSLSSNGNVTESGCKECEELEEKNIKEFLQSFVHIVQMFINTSAAAGSGATNFSLLKQAGDVEENPGPGSAPRRARGCRTLGLPALLLLLLLRPPATRGITCPPPMSVEHADIWVKSYSLYSRERYICNSGFKRKAGTSSLTECVLNKATNVAHWTTPSLKCIRDPALVHQRPAPPSTVTTAGVTPQPESLSPSGKEPAASSPSSNNTAATTAAIVPGSQLMPSKSPSTGTTEISSHESSHGTPSQTTAKNWELTASASHQPPGVYPQGHSDTTVAISTSTVLLCGLSAVSLLACYLKSRQTPPLASVEMEAMEALPVTWGTSSRDEDLENCSHHLGRSGSSGDKTHTCPPCPAPELLGGPSVFLFPPKPKDTLMISRTPEVTCVVVDVSHEDPEVKFNWYVDGVEVHNAKTKPREEQYNSTYRVVSVLTVLHQDWLNGKEYKCKVSNKALPAPIEKTISKAKGQPREPQVYTLPPSREEMTKNQVSLTCLVKGFYPSDIAVEWESNGQPENNYKTTPPVLDSDGSFFLYSKLTVDKSRWQQGNVFSCSVMHEALHNHYTQKSLSLSPGK

SEQ ID NO: 12 - DNA, 501 bp, Artificial Sequence
  Human interferon gamma
atgaaatatacaagttatatcttggcttttcagctctgcatcgttttgggttctcttggctgttactgccaggacccatatgtaaaagaagcagaaaaccttaagaaatattttaatgcaggtcattcagatgtagcggataatggaactcttttcttaggcattttgaagaattggaaagaggagagtgacagaaaaataatgcagagccaaattgtctccttttacttcaaactttttaaaaactttaaagatgaccagagcatccaaaagagtgtggagaccatcaaggaagacatgaatgtcaagtttttcaatagcaacaaaaagaaacgagatgacttcgaaaagctgactaattattcggtaactgacttgaatgtccaacgcaaagcaatacatgaactcatccaagtgatggctgaactgtcgccagcagctaaaacagggaagcgaaaaaggagtcagatgctgtttcgaggtcgaagagcatcccagtaa

SEQ ID NO: 13 - DNA, 1101 bp, Artificial Sequence
  hFlt3L-NY-ESO-1 full length
atggatgctatgaaacgaggactgtgttgtgtgttgcttctgtgtggagcggtttttgtgagtcccactcaggattgcagcttccagcattcacccatatcatcagattttgcagtaaagatcagggaactctccgattatctccttcaagactaccccgtaacagtggcctccaatttgcaagacgaagagctttgtggtgccctctggcggctcgttttggcccaaaggtggatggaacggcttaagacagtcgctggcagcaagatgcaagggttgctcgaacgagtcaatacagagatccattttgtaaccaagtgtgcatttcaaccgccgccaagctgccttcgctttgttcagacgaatataagtagactgttgcaggaaacctccgagcaactcgtagccctgaagccctggattacacggcaaaatttcagtcggtgccttgagcttcagtgtcagcctgatagtagtaccttgcctccgccatggtcccccaggcctcttgaagctacagctccgacagcccctcagccgggcagtagtggtagttctggacaagcggagggaagagggacggggggctcaacgggagacgccgatggacctggcggtcctggtatcccggacggcccaggtggcaatgctggcggtccaggcgaggctggtgcaactggtggacgcgggccgcggggcgcgggtgctgcacgggcaagtggccctgggggcggcgctcctcggggtccgcatgggggtgcagccagtggactcaatgggtgctgcagatgcggcgcgagaggtccggaaagtcgattgcttgaattttacctcgcaatgcccttcgcaacgccgatggaggctgaactggccaggcgcagtcttgcccaggacgcgcctcccttgccagtgcccggtgtgctgcttaaagagttcactgtttctggtaacatcttgacgattcgcctgacggcagcagaccatcgacaactccagctctccatctcttcatgtcttcagcagctctcactgttgatgtggatcacacagtgtttcttgcccgtgtttctcgcacagcctccatctggacagagaaggtaa

SEQ ID NO: 14 - protein, 366 aa, Artificial Sequence
  hFlt3L-NY-ESO-1 full length
MDAMKRGLCCVLLLCGAVFVSPTQDCSFQHSPISSDFAVKIRELSDYLLQDYPVTVASNLQDEELCGALWRLVLAQRWMERLKTVAGSKMQGLLERVNTEIHFVTKCAFQPPPSCLRFVQTNISRLLQETSEQLVALKPWITRQNFSRCLELQCQPDSSTLPPPWSPRPLEATAPTAPQPGSSGSSGQAEGRGTGGSTGDADGPGGPGIPDGPGGNAGGPGEAGATGGRGPRGAGAARASGPGGGAPRGPHGGAASGLNGCCRCGARGPESRLLEFYLAMPFATPMEAELARRSLAQDAPPLPVPGVLLKEFTVSGNILTIRLTAADHRQLQLSISSCLQQLSLLMWITQCFLPVFLAQPPSGQRR

SEQ ID NO: 15 - DNA, 867 bp, Artificial Sequence
  hFlt3L-NY-ESO-1 80-180aa
atggatgctatgaaacgaggactgtgttgtgtgttgcttctgtgtggagcggtttttgtgagtcccactcaggattgcagcttccagcattcacccatatcatcagattttgcagtaaagatcagggaactctccgattatctccttcaagactaccccgtaacagtggcctccaatttgcaagacgaagagctttgtggtgccctctggcggctcgttttggcccaaaggtggatggaacggcttaagacagtcgctggcagcaagatgcaagggttgctcgaacgagtcaatacagagatccattttgtaaccaagtgtgcatttcaaccgccgccaagctgccttcgctttgttcagacgaatataagtagactgttgcaggaaacctccgagcaactcgtagccctgaagccctggattacacggcaaaatttcagtcggtgccttgagcttcagtgtcagcctgatagtagtaccttgcctccgccatggtcccccaggcctcttgaagctacagctccgacagcccctcagccgggcagtagtggtagttctggagccagggggccggagagccgcctgcttgagttctacctcgccatgcctttcgcgacacccatggaagcagagctggcccgcaggagcctggcccaggatgccccaccgcttcccgtgccaggggtgcttctgaaggagttcactgtgtccggcaacatactgactatccgactgactgctgcagaccaccgccaactgcagctctccatcagctcctgtctccagcagctttccctgttgatgtggatcacgcagtgctttctgcccgtgtttttggctcagcctccctcagggcagaggcgctaa

SEQ ID NO: 16 - protein, 288 aa, Artificial Sequence
  hFlt3L-NY-ESO-1 80-180aa
MDAMKRGLCCVLLLCGAVFVSPTQDCSFQHSPISSDFAVKIRELSDYLLQDYPVTVASNLQDEELCGALWRLVLAQRWMERLKTVAGSKMQGLLERVNTEIHFVTKCAFQPPPSCLRFVQTNISRLLQETSEQLVALKPWITRQNFSRCLELQCQPDSSTLPPPWSPRPLEATAPTAPQPGSSGSSGARGPESRLLEFYLAMPFATPMEAELARRSLAQDAPPLPVPGVLLKEFTVSGNILTIRLTAADHRQLQLSISSCLQQLSLLMWITQCFLPVFLAQPPSGQRR

SEQ ID NO: 17 - DNA, 828 bp, Artificial Sequence
  hFlt3L-NY-ESO various peptides
atggatgctatgaaacgaggactgtgttgtgtgttgcttctgtgtggagcggtttttgtgagtcccactcaggattgcagcttccagcattcacccatatcatcagattttgcagtaaagatcagggaactctccgattatctccttcaagactaccccgtaacagtggcctccaatttgcaagacgaagagctttgtggtgccctctggcggctcgttttggcccaaaggtggatggaacggcttaagacagtcgctggcagcaagatgcaagggttgctcgaacgagtcaatacagagatccattttgtaaccaagtgtgcatttcaaccgccgccaagctgccttcgctttgttcagacgaatataagtagactgttgcaggaaacctccgagcaactcgtagccctgaagccctggattacacggcaaaatttcagtcggtgccttgagcttcagtgtcagcctgatagtagtaccttgcctccgccatggtcccccaggcctcttgaagctacagctccgacagcccctcagccgggcagtagtggtagttctggaaggggacctgagtcaaggctgctcgaattctacttggcaatgccttttgcgacccctatgctgcttgaattttaccttgcaatgcccttcgccacccccatggaagcagaactcgcccggcgatccttggctcagagcctcttgatgtggataactcaatgcagtttgttgatgtggataactcaatgctttctgcccgttttttggataacgcaatgctttctcccggtgtttctcgctcaaccccctagcgggcaaaggcgctaa

SEQ ID NO: 18 - protein, 275 aa, Artificial Sequence
  hFlt3L-NY-ESO various peptides
MDAMKRGLCCVLLLCGAVFVSPTQDCSFQHSPISSDFAVKIRELSDYLLQDYPVTVASNLQDEELCGALWRLVLAQRWMERLKTVAGSKMQGLLERVNTEIHFVTKCAFQPPPSCLRFVQTNISRLLQETSEQLVALKPWITRQNFSRCLELQCQPDSSTLPPPWSPRPLEATAPTAPQPGSSGSSGRGPESRLLEFYLAMPFATPMLLEFYLAMPFATPMEAELARRSLAQSLLMWITQCSLLMWITQCFLPVFWITQCFLPVFLAQPPSGQRR

SEQ ID NO: 19 - DNA, 66 bp, Artificial Sequence
  Translational modifier: Exon skipping motif P2A
ggatctggggccaccaacttttcattgctcaagcaggcgggcgatgtggaggaaaaccctggcccc

SEQ ID NO: 20 - DNA, 63 bp, Artificial Sequence
  Translational modifier: Exon skipping motif T2A
ggaagcggagagggcagaggaagtctgctaacatgcggtgacgtcgaggagaatcctggccca

SEQ ID NO: 21 - DNA, 69 bp, Artificial Sequence
  Translational modifier: Exon skipping motif E2A
ggaagcggacagtgtactaattatgctctcttgaaattggctggagatgttgagagcaaccctggacct

SEQ ID NO: 22 - DNA, 75 bp, Artificial Sequence
  Translational modifier: Exon skipping motif F2A
ggcagcggcgtgaagcagaccctgaacttcgacctgctgaagctggccggcgacgtggagagcaaccccggcccc

SEQ ID NO: 23 - DNA, 568 bp, Artificial Sequence
  Translational modifier: Internal Ribosomal Entry Sequence (IRES)
tccgcccccccccctaacgttactggccgaagccgcttggaataaggccggtgtgcgtttgtctatatgttattttccaccatattgccgtcttttggcaatgtgagggcccggaaacctggccctgtcttcttgacgagcattcctaggggtctttcccctctcgccaaaggaatgcaaggtctgttgaatgtcgtgaaggaagcagttcctctggaagcttcttgaagacaaacaacgtctgtagcgaccctttgcaggcagcggaaccccccacctggcgacaggtgcctctgcggccaaaagccacgtgtataagatacacctgcaaaggcggcacaaccccagtgccacgttgtgagttggatagttgtggaaagagtcaaatggctctcctcaagcgtattcaacaaggggctgaaggatgcccagaaggtaccccattgtatgggatctgatctggggcctcggtgcacatgctttacatgtgtttagtcgaggttaaaaaaacgtctaggccccccgaaccacggggacgtggttttcctttgaaaaacacgatgataat

SEQ ID NO: 24 - DNA, 90 bp, Artificial Sequence
  Ovalbumin aa 241-270
tccatgcttgtgttgttgcctgacgaggtgtccgggttggagcagttggaaagcataataaacttcgagaagttgactgaatggacataa

SEQ ID NO: 25 - protein, 29 aa, Artificial Sequence
  Ovalbumin aa 241-270
SMLVLLPDEVSGLEQLESIINFEKLTEWT